European Patent Application EP 4 257 678 A1, published October 11, 2023. Title: A method for producing a pluripotent stem cell population. Applicant: KANEKA CORPORATION RIKEN. The sequence listing filed with the application follows.

SEQUENCE LISTING (8 sequences)

SEQ ID NO: 1 - DNA, 21 bp, Artificial
  Synthetic DNA
cctcatgaagatcctcaccga

SEQ ID NO: 2 - DNA, 21 bp, Artificial
  Synthetic DNA
ttgccaatggtgatgacctgg

SEQ ID NO: 3 - DNA, 23 bp, Artificial
  Synthetic DNA
agtgggtggaggaagctgacaac

SEQ ID NO: 4 - DNA, 24 bp, Artificial
  Synthetic DNA
tcgttgtgcatagtcgctgcttga

SEQ ID NO: 5 - DNA, 22 bp, Artificial
  Synthetic DNA
caccaatcccatccacactcac

SEQ ID NO: 6 - DNA, 21 bp, Artificial
  Synthetic DNA
gcaaagctcctaccgtaccac

SEQ ID NO: 7 - DNA, 24 bp, Artificial
  Synthetic DNA
agcctccagcagatgcaagaactc

SEQ ID NO: 8 - DNA, 24 bp, Artificial
  Synthetic DNA
ttgctccacattggaaggttccca